European Patent Application EP 4 538 291 A1, published April 16, 2025. Title: Anti-nectin-4 antibody, and antibody drug conjugate and use thereof. Applicant: Bio-Thera Solutions, Ltd. The sequence listing filed with the application follows.

SEQUENCE LISTING (20 sequences)

SEQ ID NO: 1 - protein, 344 aa, synthetic construct
MKWVTFISLLFLFSSAYSGELETSDVVTVVLGQDAKLPCFYRGDSGEQVGQVAWARVDAGEGAQELALLHSKYGLHVSPAYEGRVEQPPPPRNPLDGSVLLRNAVQADEGEYECRVSTFPAGSFQARLRLRVLVPPLPSLNPGPALEEGQGLTLAASCTAEGSPAPSVTWDTEVKGTTSSRSFKHSRSAAVTSEFHLVPSRSMNGQPLTCVVSHPGLLQDQRITHILHVSFLAEASVRGLEDQNLWHIGREGAMLKCLSEGQPPPSYNWTRLDGPLPSGVRVDGDTLGFPPLTTEHSGIYVCHVSNEFSSRDSQVTVDVLDPQEDSGKQVDLVSASHHHHHHHH

SEQ ID NO: 2 - protein, 8 aa, synthetic construct
GFTFSSYN

SEQ ID NO: 3 - protein, 10 aa, synthetic construct
YISSSSSTIY

SEQ ID NO: 4 - protein, 8 aa, synthetic construct
AYYYGMDV

SEQ ID NO: 5 - protein, 11 aa, synthetic construct
RASQGISGWLA

SEQ ID NO: 6 - protein, 7 aa, synthetic construct
AASTLQS

SEQ ID NO: 7 - protein, 9 aa, synthetic construct
GPGWVFGQG

SEQ ID NO: 8 - protein, 117 aa, synthetic construct
EVQLVESGGGLVQPGGSLRLSCAASGFTFSSYNMNWVRQAPGKGLEWVSYISSSSSTIYYADSVKGRFTISRDNAKNSLSLQMNSLRDEDTAVYYCARAYYYGMDVWGQGTLVTVSS

SEQ ID NO: 9 - protein, 330 aa, synthetic construct [sequence omitted]

SEQ ID NO: 10 - protein, 107 aa, synthetic construct
DIQMTQSPSSVSASVGDRVTITCRASQGISGWLAWYQQKPGKAPKFLIYAASTLQSGVPSRFSGSGSGTDFTLTISSLQPEDFATYYCQQAGPGWVFGQGTKVEIKR

SEQ ID NO: 11 - protein, 106 aa, synthetic construct
TVAAPSVFIFPPSDEQLKSGTASVVCLLNNFYPREAKVQWKVDNALQSGNSQESVTEQDSKDSTYSLSSTLTLSKADYEKHKVYACEVTHQGLSSPVTKSFNRGEC

SEQ ID NO: 12 - protein, 447 aa, synthetic construct
EVQLVESGGGLVQPGGSLRLSCAASGFTFSSYNMNWVRQAPGKGLEWVSYISSSSSTIYYADSVKGRFTISRDNAKNSLSLQMNSLRDEDTAVYYCARAYYYGMDVWGQGTLVTVSSASTKGPSVFPLAPSSKSTSGGTAALGCLVKDYFPEPVTVSWNSGALTSGVHTFPAVLQSSGLYSLSSVVTVPSSSLGTQTYICNVNHKPSNTKVDKKVEPKSCDKTHTCPPCPAPELLGGPSVFLFPPKPKDTLMISRTPEVTCVVVDVSHEDPEVKFNWYVDGVEVHNAKTKPREEQYNSTYRVVSVLTVLHQDWLNGKEYKCKVSNKALPAPIEKTISKAKGQPREPQVYTLPPSRDELTKNQVSLTCLVKGFYPSDIAVEWESNGQPENNYKTTPPVLDSDGSFFLYSKLTVDKSRWQQGNVFSCSVMHEALHNHYTQKSLSLSPGK

SEQ ID NO: 13 - DNA, 1344 bp, synthetic construct
  source 1..1344: mol_type = other DNA
gaggtgcagctggtggagtccggcggcggactggtgcagcctggaggaagcctgaggctgtcctgtgccgcctccggcttcacattctccagctacaatatgaactgggtgagacaggcccccggcaagggcctggagtgggttagctacatcagctccagctccagcacaatctactacgccgacagcgtgaagggcagattcactatctccagggacaatgccaagaatagcctgtccctgcagatgaattccctgagagatgaggacacagccgtgtactactgtgccagggcctactactacggcatggacgtgtggggccagggtaccctggttaccgttagcagcgcctctaccaagggcccctctgtgtttcctctggctccctccagcaagtctacctctggtggaacagctgccctgggctgcctggtcaaggattactttcctgagcctgtcaccgtgtcctggaactctggcgctctgacatctggcgtgcacacctttccagctgtgctccagtcctccggcctgtactctctgtcctctgtcgtgaccgtgccttctagctctctgggcacccagacctacatctgcaatgtgaaccacaagccttccaacaccaaggtggacaagaaggtggaacccaagtcctgcgacaagacccacacctgtcctccatgtcctgctccagaactgctcggcggaccttccgtgttcctgtttcctccaaagcctaaggacaccctgatgatctctcggacccctgaagtgacctgcgtggtggtggatgtgtctcacgaagatcccgaagtgaagttcaactggtacgtggacggcgtggaagtgcacaacgccaagaccaagcctagagaggaacagtacaactccacctacagagtggtgtccgtgctgaccgtgctgcaccaggattggctgaacggcaaagagtacaagtgcaaggtgtccaacaaggccctgcctgctcctatcgaaaagaccatctccaaggccaagggccagcctagggaaccccaggtttacaccttgcctccatctcgggacgagctgaccaagaaccaggtgtccctgacctgtctcgtgaagggcttctacccctccgacatcgccgtggaatgggagtctaatggccagcctgagaacaactacaagacaacccctcctgtgctggactccgacggctcattcttcctgtactccaagctgacagtggacaagtccagatggcagcagggcaacgtgttctcctgctccgtgatgcacgaggccctgcacaatcactacacccagaagtccctgtctctgtcccctggcaaataa

SEQ ID NO: 14 - protein, 213 aa, synthetic construct
DIQMTQSPSSVSASVGDRVTITCRASQGISGWLAWYQQKPGKAPKFLIYAASTLQSGVPSRFSGSGSGTDFTLTISSLQPEDFATYYCQQAGPGWVFGQGTKVEIKRTVAAPSVFIFPPSDEQLKSGTASVVCLLNNFYPREAKVQWKVDNALQSGNSQESVTEQDSKDSTYSLSSTLTLSKADYEKHKVYACEVTHQGLSSPVTKSFNRGEC

SEQ ID NO: 15 - DNA, 642 bp, synthetic construct
  source 1..642: mol_type = other DNA
gacatccagatgacacagagccccagcagcgtgtccgcctccgtgggagatagagtgacaatcacatgtagagccagccagggcatcagcggctggctggcttggtaccagcagaagcccggcaaggcccccaagttcctgatctacgccgccagcacactgcagtccggcgtgccttccaggttttccggcagcggctccggcacagactttaccctgacaatcagcagcctgcagcctgaggatttcgccacatactactgccagcaggccggccccggctgggttttcggacagggaacaaaggtggagatcaagcgtacggtggctgcaccatctgtcttcatcttcccgccatctgatgagcagttgaaatctggaactgcctctgttgtgtgcctgctgaataacttctatcccagagaggccaaagtacagtggaaggtggataacgccctccaatcgggtaactcccaggagagtgtcacagagcaggacagcaaggacagcacctacagcctcagcagcaccctgacgctgagcaaagcagactacgagaaacacaaagtctacgcctgcgaagtcacccatcagggcctgagctcgcccgtcacaaagagcttcaacaggggagagtgttga

SEQ ID NO: 16 - DNA, 66 bp, synthetic construct
  source 1..66: mol_type = other DNA
atggacatgagagtgcctgcccagctgctgggcctgctgctgctgtggttccctggcagcagatgc

SEQ ID NO: 17 - protein, 214 aa, synthetic construct
DIQMTQSPSSVSASVGDRVTITCRASQGISGWLAWYQQKPGKAPKFLIYAASTLQSGVPSRFSGSGSGTDFTLTISSLQPEDFATYYCQQANSFPPTFGGGTKVEIKRTVAAPSVFIFPPSDEQLKSGTASVVCLLNNFYPREAKVQWKVDNALQSGNSQESVTEQDSKDSTYSLSSTLTLSKADYEKHKVYACEVTHQGLSSPVTKSFNRGEC

SEQ ID NO: 18 - protein, 19 aa, synthetic construct
MELGLCWVFLVAILEGVQC

SEQ ID NO: 19 - DNA, 57 bp, synthetic construct
  source 1..57: mol_type = other DNA
atggagctgggcctgtgttgggtgtttctggtggccatcctggagggcgtgcagtgc

SEQ ID NO: 20 - protein, 22 aa, synthetic construct
MDMRVPAQLLGLLLLWFPGSRC